European Patent Application EP 4 215 546 A1, published July 26, 2023. Title: Anti-Nectin-4 antibody, conjugate including same, and application thereof. Applicant: SICHUAN KELUN-BIOTECH BIOPHARMACEUTICAL CO., LTD. The sequence listing filed with the application follows.

SEQUENCE LISTING (64 sequences)

SEQ ID NO: 1 - protein, 120 aa, Artificial Sequence
  31#VH
EVQLQQPGADLVRPGASVKLSCKASGYTFTDYWMNWVKLRPGQGLEWIGMIHPSDSETRLNQKFKDKATLTVDKSSSTAYMQLSSPTSEDSAVYYCARWDFRIYYAMDYWGQGTSVTVSS

SEQ ID NO: 2 - protein, 113 aa, Artificial Sequence
  31#VL
DVVITQSPSSLAMSVGQKVTMSCKSSQSLLNTNSQKNYLAWYQQKPGQSPKLLVYFASTRESGVPDRFIGSGSGTDFTLTITSVQAEDLADYFCQQHYSTPLTFGAGTKLEIK

SEQ ID NO: 3 - protein, 7 aa, Artificial Sequence
  Chothia  31#/31HZ  CDR-H1
GYTFTDY

SEQ ID NO: 4 - protein, 6 aa, Artificial Sequence
  Chothia  31# /31HZ CDR-H2
HPSDSE

SEQ ID NO: 5 - protein, 11 aa, Artificial Sequence
  Chothia/Abm/ Kabat  31# /31HZ  CDR-H3
WDFRIYYAMDY

SEQ ID NO: 6 - protein, 17 aa, Artificial Sequence
  Chothia/Abm/ Kabat  31# /31HZ CDR-L1
KSSQSLLNTNSQKNYLA

SEQ ID NO: 7 - protein, 7 aa, Artificial Sequence
  Chothia/Abm/ Kabat  31#  /31HZ CDR-L2
FASTRES

SEQ ID NO: 8 - protein, 9 aa, Artificial Sequence
  Chothia/Abm/ Kabat/IMGT 31#/31HZ/74#/74HZ CDR-L3
QQHYSTPLT

SEQ ID NO: 9 - protein, 10 aa, Artificial Sequence
  Abm  31#/31HZ CDR-H1
GYTFTDYWMN

SEQ ID NO: 10 - protein, 10 aa, Artificial Sequence
  Abm  31#  /31HZ CDR-H2
MIHPSDSETR

SEQ ID NO: 11 - protein, 5 aa, Artificial Sequence
  Kabat  31#  /31HZ CDR-H1
DYWMN

SEQ ID NO: 12 - protein, 17 aa, Artificial Sequence
  Kabat  31# CDR-H2
MIHPSDSETRLNQKFKD

SEQ ID NO: 13 - protein, 8 aa, Artificial Sequence
  IMGT  31# /31HZ  CDR-H1
GYTFTDYW

SEQ ID NO: 14 - protein, 8 aa, Artificial Sequence
  IMGT  31#/31HZ  CDR-H2
IHPSDSET

SEQ ID NO: 15 - protein, 13 aa, Artificial Sequence
  IMGT  31# /31HZ  CDR-H3
ARWDFRIYYAMDY

SEQ ID NO: 16 - protein, 12 aa, Artificial Sequence
  IMGT  31# /31HZ  CDR-L1
QSLLNTNSQKNY

SEQ ID NO: 17 - protein, 3 aa, Artificial Sequence
  IMGT  31# /31HZ CDR-L2
FAS

SEQ ID NO: 18 - protein, 10 aa, Artificial Sequence
  Chothia  56HZ  CDR-H1
GYFNSITSDY

SEQ ID NO: 19 - protein, 117 aa, Artificial Sequence
  56#VH
QVQLKESGPGLVKPSQSLSLTCTVTGYSITSDYDWHWIRHFPGNMLEWMGYISFSGRTYYNPSLKSRISITHDTSKNHFFLRLNSVTTEDTATYYCARGNYDGFDYWGQGTTLTVSS

SEQ ID NO: 20 - protein, 108 aa, Artificial Sequence
  56#VL
DIQLTQSPAILSVSPGERVSFSCRASQNIGTSIHWYQHRTNGSPRLLIKFASESISGIPSRFSGSGSGTDFTLSINSVESEDIADYYCQQSKSWPTYTFGGGTKLEIK

SEQ ID NO: 21 - protein, 8 aa, Artificial Sequence
  Chothia  56# CDR-H1
GYSITSDY

SEQ ID NO: 22 - protein, 5 aa, Artificial Sequence
  Chothia  56#/56HZ  CDR-H2
SFSGR

SEQ ID NO: 23 - protein, 8 aa, Artificial Sequence
  Chothia/Abm/ Kabat  56#  /56HZ  CDR-H3
GNYDGFDY

SEQ ID NO: 24 - protein, 11 aa, Artificial Sequence
  Chothia/Abm/ Kabat  56# /56HZ   CDR-L1
RASQNIGTSIH

SEQ ID NO: 25 - protein, 7 aa, Artificial Sequence
  Chothia/Abm/ Kabat  56# /56HZ  CDR-L2
FASESIS

SEQ ID NO: 26 - protein, 10 aa, Artificial Sequence
  Chothia/Abm/ Kabat/IMGT  56#/56HZ   CDR-L3
QQSKSWPTYT

SEQ ID NO: 27 - protein, 11 aa, Artificial Sequence
  Abm  56# CDR-H1
GYSITSDYDWH

SEQ ID NO: 28 - protein, 9 aa, Artificial Sequence
  Abm  56# /56HZ  CDR-H2
YISFSGRTY

SEQ ID NO: 29 - protein, 6 aa, Artificial Sequence
  Kabat  56# CDR-H1
SDYDWH

SEQ ID NO: 30 - protein, 16 aa, Artificial Sequence
  Kabat  56#/56HZ   CDR-H2
YISFSGRTYYNPSLKS

SEQ ID NO: 31 - protein, 9 aa, Artificial Sequence
  IMGT  56# CDR-H1
GYSITSDYD

SEQ ID NO: 32 - protein, 7 aa, Artificial Sequence
  IMGT  56#/56HZ   CDR-H2
ISFSGRT

SEQ ID NO: 33 - protein, 10 aa, Artificial Sequence
  IMGT  56# /56HZ   CDR-H3
ARGNYDGFDY

SEQ ID NO: 34 - protein, 6 aa, Artificial Sequence
  IMGT  56# /56HZ  CDR-L1
QNIGTS

SEQ ID NO: 35 - protein, 3 aa, Artificial Sequence
  IMGT  56#/56HZ   CDR-L2
FAS

SEQ ID NO: 36 - protein, 13 aa, Artificial Sequence
  Abm  56HZ  CDR-H1
GYFNSITSDYDWH

SEQ ID NO: 37 - protein, 124 aa, Artificial Sequence
  74#VH
EVQLQQPGAELVRPGASVKLSCKASGYTFINYWMNWVKQRPGQGLEWIGMIHPSDSATRLNQKFKDKATLTVDKSSSTAYMQLSSPTSEDSAVYYCARWGNFYTVNAWYYFDYWGHGTTLTVSS

SEQ ID NO: 38 - protein, 113 aa, Artificial Sequence
  74#VL
DIVITQSPSSLAMSVGQKVTMSCKSSQTLLNSNTQKNYLAWYQQKPGQSPKLLFYFASTRESGVPDRFIGSGSGTNFTLTISSVQAEDLADYFCQQHYSTPLTFGAGTKLEIK

SEQ ID NO: 39 - protein, 7 aa, Artificial Sequence
  Chothia  74#/74HZ  CDR-H1
GYTFINY

SEQ ID NO: 40 - protein, 6 aa, Artificial Sequence
  Chothia  74#/74HZ  CDR-H2
HPSDSA

SEQ ID NO: 41 - protein, 15 aa, Artificial Sequence
  Chothia/Abm/ Kabat 74#/74HZ  CDR-H3
WGNFYTVNAWYYFDY

SEQ ID NO: 42 - protein, 17 aa, Artificial Sequence
  Chothia/Abm/ Kabat  74#/74HZ  CDR-L1
KSSQTLLNSNTQKNYLA

SEQ ID NO: 43 - protein, 7 aa, Artificial Sequence
  Chothia/Abm/ Kabat  74#/74HZ  CDR-L2
FASTRES

SEQ ID NO: 44 - protein, 8 aa, Artificial Sequence
  Kabat  56HZ  CDR-H1
ITSDYDWH

SEQ ID NO: 45 - protein, 10 aa, Artificial Sequence
  Abm  74#/74HZ  CDR-H1
GYTFINYWMN

SEQ ID NO: 46 - protein, 10 aa, Artificial Sequence
  Abm  74#/74HZ  CDR-H2
MIHPSDSATR

SEQ ID NO: 47 - protein, 5 aa, Artificial Sequence
  Kabat  74#  /74HZ CDR-H1
NYWMN

SEQ ID NO: 48 - protein, 17 aa, Artificial Sequence
  Kabat  74# CDR-H2
MIHPSDSATRLNQKFKD

SEQ ID NO: 49 - protein, 8 aa, Artificial Sequence
  IMGT  74#/74HZ  CDR-H1
GYTFINYW

SEQ ID NO: 50 - protein, 8 aa, Artificial Sequence
  IMGT  74#/74HZ CDR-H2
IHPSDSAT

SEQ ID NO: 51 - protein, 17 aa, Artificial Sequence
  IMGT  74#/74HZ CDR-H3
ARWGNFYTVNAWYYFDY

SEQ ID NO: 52 - protein, 12 aa, Artificial Sequence
  IMGT  74#/74HZ  CDR-L1
QTLLNSNTQKNY

SEQ ID NO: 53 - protein, 3 aa, Artificial Sequence
  IMGT  74#/74HZ CDR-L2
FAS

SEQ ID NO: 54 - protein, 11 aa, Artificial Sequence
  IMGT  56HZ  CDR-H1
GYFNSITSDYD

SEQ ID NO: 55 - protein, 120 aa, Artificial Sequence
  31HZ  VH
QVQLVQSGAEVKKPGSSVKVSCKASGYTFTDYWMNWVRLAPGQGLEWIGMIHPSDSETRLNQKFQGRVTLTVDKSTSTAYMELSSLRSEDTAVYYCARWDFRIYYAMDYWGQGTLVTVSS

SEQ ID NO: 56 - protein, 113 aa, Artificial Sequence
  31HZ  VL
DVVITQSPDSLAVSLGERATINCKSSQSLLNTNSQKNYLAWYQQKPGQSPKLLVYFASTRESGVPDRFSGSGSGTDFTLTISSLQAEDVAVYFCQQHYSTPLTFGGGTKVEIK

SEQ ID NO: 57 - protein, 119 aa, Artificial Sequence
  56HZ  VH
QVQLQESGPGLVKPSQTLSLTCTVSGYFNSITSDYDWHWIRHHPGKGLEWMGYISFSGRTYYNPSLKSRVTISHDTSKNQFSLKLSSVTAADTAVYYCARGNYDGFDYWGQGTLVTVSS

SEQ ID NO: 58 - protein, 108 aa, Artificial Sequence
  56HZ  VL
DIVLTQSPATLSLSPGERATLSCRASQNIGTSIHWYQHKPGQSPRLLIKFASESISGIPARFSGSGSGTDFTLTISSLEPEDFAVYYCQQSKSWPTYTFGGGTKVEIK

SEQ ID NO: 59 - protein, 124 aa, Artificial Sequence
  74HZ  VH
QVQLVQSGAEVKKPGSSVKVSCKASGYTFINYWMNWVRQAPGQGLEWIGMIHPSDSATRLNQSFQGRVTLTVDKSTSTAYMELSSLRSEDTAVYYCARWGNFYTVNAWYYFDYWGQGTLVTVSS

SEQ ID NO: 60 - protein, 113 aa, Artificial Sequence
  74HZ  VL
DIVITQSPDSLAVSLGERATINCKSSQTLLNSNTQKNYLAWYQQKPGQSPKLLFYFASTRESGVPDRFSGSGSGTDFTLTISSLQAEDVAVYFCQQHYSTPLTFGQGTKLEIK

SEQ ID NO: 61 - protein, 330 aa, Artificial Sequence [sequence omitted]

SEQ ID NO: 62 - protein, 107 aa, Artificial Sequence [sequence omitted]

SEQ ID NO: 63 - protein, 17 aa, Artificial Sequence
  Kabat  31HZ CDR-H2
MIHPSDSETRLNQKFQG

SEQ ID NO: 64 - protein, 17 aa, Artificial Sequence
  Kabat 74HZ CDR-H2
MIHPSDSATRLNQSFQG